European Patent Application EP 4 455 160 A1, published October 30, 2024. Title: 治疗血小板减少的产品及方法. Applicant: 上海循曜生物科技有限公司. Application CN. The sequence listing filed with the application follows.

SEQUENCE LISTING (21 sequences)

SEQ ID NO: 1 - DNA, 933 bp, Homo sapiens
  source 1..933: mol_type = other DNA
atggccctgcccgtgaccgccctgctgctgcccctggccctgctgctgcacgccgcccgcccccaccccatctgtgaggtctccaaagtggccagccacctagaagtgaactgtgacaagaggaatctgacagcgctgcctccagacctgccgaaagacacaaccatcctccacctgagtgagaacctcctgtacaccttctccctggcaaccctgatgccttacactcgcctcactcagctgaacctagataggtgcgagctcaccaagctccaggtcgatgggacgctgccagtgctggggaccctggatctatcccacaatcagctgcaaagcctgcccttgctagggcagacactgcctgctctcaccgtcctggacgtctccttcaaccggctgacctcgctgcctcttggtgccctgcgtggtcttggcgaactccaagagctctacctgaaaggcaatgagctgaagaccctgcccccagggctcctgacgcccacacccaagctggagaagctcagtctggctaacaacaacttgactgagctccccgctgggctcctgaatgggctggagaatctcgacacccttctcctccaagagaactcgctgtatacaataccaaagggcttttttgggtcccacctcctgccttttgcttttctccacgggaacccctggttatgcaactgtgagatcctctattttcgtcgctggctgcaggacaatgctgaaaatgtctacgtatggaagcaaggtgtggacgtcaaggccatgacctctaacgtggccagtgtgcagtgtgacaattcagacaagtttcccgtctacaaatacccaggaaaggggtgccccacccttggtgatgaaggtgacacagacctatatgattactacccagaagaggacactgagggcgataaggtgcgt

SEQ ID NO: 2 - protein, 290 aa, Homo sapiens
HPICEVSKVASHLEVNCDKRNLTALPPDLPKDTTILHLSENLLYTFSLATLMPYTRLTQLNLDRCELTKLQVDGTLPVLGTLDLSHNQLQSLPLLGQTLPALTVLDVSFNRLTSLPLGALRGLGELQELYLKGNELKTLPPGLLTPTPKLEKLSLANNNLTELPAGLLNGLENLDTLLLQENSLYTIPKGFFGSHLLPFAFLHGNPWLCNCEILYFRRWLQDNAENVYVWKQGVDVKAMTSNVASVQCDNSDKFPVYKYPGKGCPTLGDEGDTDLYDYYPEEDTEGDKVR

SEQ ID NO: 3 - DNA, 513 bp, Homo sapiens
  source 1..513: mol_type = other DNA
atggccctgcccgtgaccgccctgctgctgcccctggccctgctgctgcacgccgcccgcccccccacccttggtgatgaaggtgacacagacctatatgattactacccagaagaggacactgagggcgataaggtgcgtgccacaaggactgtggtcaagttccccaccaaagcccatacaaccccctggggtctattctactcatggtccactgcttctctagacagccaaatgccctcctccttgcatccaacacaagaatccactaaggagcagaccacattcccacctagatggaccccaaatttcacacttcacatggaatccatcacattctccaaaactccaaaatccactactgaaccaaccccaagcccgaccacctcagagcccgtcccggagcccgccccaaacatgaccaccctggagcccactccaagcccgaccaccccagagcccacctcagagcccgcccccagcccgaccaccccggagcccacctcagagccc

SEQ ID NO: 4 - protein, 150 aa, Homo sapiens
PTLGDEGDTDLYDYYPEEDTEGDKVRATRTVVKFPTKAHTTPWGLFYSWSTASLDSQMPSSLHPTQESTKEQTTFPPRWTPNFTLHMESITFSKTPKSTTEPTPSPTTSEPVPEPAPNMTTLEPTPSPTTPEPTSEPAPSPTTPEPTSEP

SEQ ID NO: 5 - DNA, 798 bp, Homo sapiens
  source 1..798: mol_type = other DNA
atggccctgcccgtgaccgccctgctgctgcccctggccctgctgctgcacgccgcccgcccccccacccttggtgatgaaggtgacacagacctatatgattactacccagaagaggacactgagggcgataaggtgcgtgccacaaggactgtggtcaagttccccaccaaagcccatacaaccccctggggtctattctactcatggtccactgcttctctagacagccaaatgccctcctccttgcatccaacacaagaatccactaaggagcagaccacattcccacctagatggaccccaaatttcacacttcacatggaatccatcacattctccaaaactccaaaatccactactgaaccaaccccaagcccgaccacctcagagcccgtcccggagcccgccccaaacatgaccaccctggagcccactccaagcccgaccaccccagagcccacctcagagcccgcccccagcccgaccaccccggagcccacctcagagcccgcccccagcccgaccaccccagagcccacctcagagcccgcccccagcccgaccaccccggagcccaccccaatcccgaccatcgccacaagcccgaccatcctggtgtctgccacaagcctgatcactccaaaaagcacatttttaactaccacaaaacccgtatcactcttagaatccaccaaaaaaaccatccctgaacttgatcagccaccaaagctccgtggggtgctccaagggcatttggagagctccagaaatgacccttttctccaccccgacttt

SEQ ID NO: 6 - protein, 245 aa, Homo sapiens
PTLGDEGDTDLYDYYPEEDTEGDKVRATRTVVKFPTKAHTTPWGLFYSWSTASLDSQMPSSLHPTQESTKEQTTFPPRWTPNFTLHMESITFSKTPKSTTEPTPSPTTSEPVPEPAPNMTTLEPTPSPTTPEPTSEPAPSPTTPEPTSEPAPSPTTPEPTSEPAPSPTTPEPTPIPTIATSPTILVSATSLITPKSTFLTTTKPVSLLESTKKTIPELDQPPKLRGVLQGHLESSRNDPFLHPDF

SEQ ID NO: 7 - DNA, 1590 bp, Homo sapiens
  source 1..1590: mol_type = other DNA
atggccctgcccgtgaccgccctgctgctgcccctggccctgctgctgcacgccgcccgcccccaccccatctgtgaggtctccaaagtggccagccacctagaagtgaactgtgacaagaggaatctgacagcgctgcctccagacctgccgaaagacacaaccatcctccacctgagtgagaacctcctgtacaccttctccctggcaaccctgatgccttacactcgcctcactcagctgaacctagataggtgcgagctcaccaagctccaggtcgatgggacgctgccagtgctggggaccctggatctatcccacaatcagctgcaaagcctgcccttgctagggcagacactgcctgctctcaccgtcctggacgtctccttcaaccggctgacctcgctgcctcttggtgccctgcgtggtcttggcgaactccaagagctctacctgaaaggcaatgagctgaagaccctgcccccagggctcctgacgcccacacccaagctggagaagctcagtctggctaacaacaacttgactgagctccccgctgggctcctgaatgggctggagaatctcgacacccttctcctccaagagaactcgctgtatacaataccaaagggcttttttgggtcccacctcctgccttttgcttttctccacgggaacccctggttatgcaactgtgagatcctctattttcgtcgctggctgcaggacaatgctgaaaatgtctacgtatggaagcaaggtgtggacgtcaaggccatgacctctaacgtggccagtgtgcagtgtgacaattcagacaagtttcccgtctacaaatacccaggaaaggggtgccccacccttggtgatgaaggtgacacagacctatatgattactacccagaagaggacactgagggcgataaggtgcgtgccacaaggactgtggtcaagttccccaccaaagcccatacaaccccctggggtctattctactcatggtccactgcttctctagacagccaaatgccctcctccttgcatccaacacaagaatccactaaggagcagaccacattcccacctagatggaccccaaatttcacacttcacatggaatccatcacattctccaaaactccaaaatccactactgaaccaaccccaagcccgaccacctcagagcccgtcccggagcccgccccaaacatgaccaccctggagcccactccaagcccgaccaccccagagcccacctcagagcccgcccccagcccgaccaccccggagcccacctcagagcccgcccccagcccgaccaccccagagcccacctcagagcccgcccccagcccgaccaccccggagcccaccccaatcccgaccatcgccacaagcccgaccatcctggtgtctgccacaagcctgatcactccaaaaagcacatttttaactaccacaaaacccgtatcactcttagaatccaccaaaaaaaccatccctgaacttgatcagccaccaaagctccgtggggtgctccaagggcatttggagagctccagaaatgacccttttctccaccccgacttt

SEQ ID NO: 8 - protein, 509 aa, Homo sapiens
HPICEVSKVASHLEVNCDKRNLTALPPDLPKDTTILHLSENLLYTFSLATLMPYTRLTQLNLDRCELTKLQVDGTLPVLGTLDLSHNQLQSLPLLGQTLPALTVLDVSFNRLTSLPLGALRGLGELQELYLKGNELKTLPPGLLTPTPKLEKLSLANNNLTELPAGLLNGLENLDTLLLQENSLYTIPKGFFGSHLLPFAFLHGNPWLCNCEILYFRRWLQDNAENVYVWKQGVDVKAMTSNVASVQCDNSDKFPVYKYPGKGCPTLGDEGDTDLYDYYPEEDTEGDKVRATRTVVKFPTKAHTTPWGLFYSWSTASLDSQMPSSLHPTQESTKEQTTFPPRWTPNFTLHMESITFSKTPKSTTEPTPSPTTSEPVPEPAPNMTTLEPTPSPTTPEPTSEPAPSPTTPEPTSEPAPSPTTPEPTSEPAPSPTTPEPTPIPTIATSPTILVSATSLITPKSTFLTTTKPVSLLESTKKTIPELDQPPKLRGVLQGHLESSRNDPFLHPDF

SEQ ID NO: 9 - DNA, 1305 bp, Homo sapiens
  source 1..1305: mol_type = other DNA
atggccctgcccgtgaccgccctgctgctgcccctggccctgctgctgcacgccgcccgcccccaccccatctgtgaggtctccaaagtggccagccacctagaagtgaactgtgacaagaggaatctgacagcgctgcctccagacctgccgaaagacacaaccatcctccacctgagtgagaacctcctgtacaccttctccctggcaaccctgatgccttacactcgcctcactcagctgaacctagataggtgcgagctcaccaagctccaggtcgatgggacgctgccagtgctggggaccctggatctatcccacaatcagctgcaaagcctgcccttgctagggcagacactgcctgctctcaccgtcctggacgtctccttcaaccggctgacctcgctgcctcttggtgccctgcgtggtcttggcgaactccaagagctctacctgaaaggcaatgagctgaagaccctgcccccagggctcctgacgcccacacccaagctggagaagctcagtctggctaacaacaacttgactgagctccccgctgggctcctgaatgggctggagaatctcgacacccttctcctccaagagaactcgctgtatacaataccaaagggcttttttgggtcccacctcctgccttttgcttttctccacgggaacccctggttatgcaactgtgagatcctctattttcgtcgctggctgcaggacaatgctgaaaatgtctacgtatggaagcaaggtgtggacgtcaaggccatgacctctaacgtggccagtgtgcagtgtgacaattcagacaagtttcccgtctacaaatacccaggaaaggggtgccccacccttggtgatgaaggtgacacagacctatatgattactacccagaagaggacactgagggcgataaggtgcgtgccacaaggactgtggtcaagttccccaccaaagcccatacaaccccctggggtctattctactcatggtccactgcttctctagacagccaaatgccctcctccttgcatccaacacaagaatccactaaggagcagaccacattcccacctagatggaccccaaatttcacacttcacatggaatccatcacattctccaaaactccaaaatccactactgaaccaaccccaagcccgaccacctcagagcccgtcccggagcccgccccaaacatgaccaccctggagcccactccaagcccgaccaccccagagcccacctcagagcccgcccccagcccgaccaccccggagcccacctcagagccc

SEQ ID NO: 10 - protein, 414 aa, Homo sapiens
HPICEVSKVASHLEVNCDKRNLTALPPDLPKDTTILHLSENLLYTFSLATLMPYTRLTQLNLDRCELTKLQVDGTLPVLGTLDLSHNQLQSLPLLGQTLPALTVLDVSFNRLTSLPLGALRGLGELQELYLKGNELKTLPPGLLTPTPKLEKLSLANNNLTELPAGLLNGLENLDTLLLQENSLYTIPKGFFGSHLLPFAFLHGNPWLCNCEILYFRRWLQDNAENVYVWKQGVDVKAMTSNVASVQCDNSDKFPVYKYPGKGCPTLGDEGDTDLYDYYPEEDTEGDKVRATRTVVKFPTKAHTTPWGLFYSWSTASLDSQMPSSLHPTQESTKEQTTFPPRWTPNFTLHMESITFSKTPKSTTEPTPSPTTSEPVPEPAPNMTTLEPTPSPTTPEPTSEPAPSPTTPEPTSEP

SEQ ID NO: 11 - protein, 513 aa, synthetic construct
HPICEVSKVASHLEVNCDKRNLTALPPDLPKDTTILHLSENLLYTFSLATLMPYTRLTQLNLDRCELTKLQVDGTLPVLGTLDLSHNQLQSLPLLGQTLPALTVLDVSFNRLTSLPLGALRGLGELQELYLKGNELKTLPPGLLTPTPKLEKLSLANNNLTELPAGLLNGLENLDTLLLQENSLYTIPKGFFGSHLLPFAFLHGNPWLCNCEILYFRRWLQDNAENVYVWKQKVDVKAMTSNVASVQCDNSDKFPVYKYPGKGCPTLGDEGDTDLYDYYPEEDTEGDKVRTTTPAPRPPTPAPTIASQPLSLRPEACRPAAGGAVHTRGLDFACDIYIWAPLAGTCGVLLLSLVITLYCKRGRKKLLYIFKQPFMRPVQTTQEEDGCSCRFPEEEEGGCELRVKFSRSADAPAYQQGQNQLYNELNLGRREEYDVLDKRRGRDPEMGGKPRRKNPQEGLYNELQKDKMAEAYSEIGMKGERRRGKGHDGLYQGLSTATKDTYDALHMQALPPR

SEQ ID NO: 12 - protein, 373 aa, synthetic construct
PTLGDEGDTDLYDYYPEEDTEGDKVRATRTVVKFPTKAHTTPWGLFYSWSTASLDSQMPSSLHPTQESTKEQTTFPPRWTPNFTLHMESITFSKTPKSTTEPTPSPTTSEPVPEPAPNMTTLEPTPSPTTPEPTSEPAPSPTTPEPTSEPTTTPAPRPPTPAPTIASQPLSLRPEACRPAAGGAVHTRGLDFACDIYIWAPLAGTCGVLLLSLVITLYCKRGRKKLLYIFKQPFMRPVQTTQEEDGCSCRFPEEEEGGCELRVKFSRSADAPAYQQGQNQLYNELNLGRREEYDVLDKRRGRDPEMGGKPRRKNPQEGLYNELQKDKMAEAYSEIGMKGERRRGKGHDGLYQGLSTATKDTYDALHMQALPPR

SEQ ID NO: 13 - protein, 468 aa, synthetic construct
PTLGDEGDTDLYDYYPEEDTEGDKVRATRTVVKFPTKAHTTPWGLFYSWSTASLDSQMPSSLHPTQESTKEQTTFPPRWTPNFTLHMESITFSKTPKSTTEPTPSPTTSEPVPEPAPNMTTLEPTPSPTTPEPTSEPAPSPTTPEPTSEPAPSPTTPEPTSEPAPSPTTPEPTPIPTIATSPTILVSATSLITPKSTFLTTTKPVSLLESTKKTIPELDQPPKLRGVLQGHLESSRNDPFLHPDFTTTPAPRPPTPAPTIASQPLSLRPEACRPAAGGAVHTRGLDFACDIYIWAPLAGTCGVLLLSLVITLYCKRGRKKLLYIFKQPFMRPVQTTQEEDGCSCRFPEEEEGGCELRVKFSRSADAPAYQQGQNQLYNELNLGRREEYDVLDKRRGRDPEMGGKPRRKNPQEGLYNELQKDKMAEAYSEIGMKGERRRGKGHDGLYQGLSTATKDTYDALHMQALPPR

SEQ ID NO: 14 - protein, 732 aa, synthetic construct
HPICEVSKVASHLEVNCDKRNLTALPPDLPKDTTILHLSENLLYTFSLATLMPYTRLTQLNLDRCELTKLQVDGTLPVLGTLDLSHNQLQSLPLLGQTLPALTVLDVSFNRLTSLPLGALRGLGELQELYLKGNELKTLPPGLLTPTPKLEKLSLANNNLTELPAGLLNGLENLDTLLLQENSLYTIPKGFFGSHLLPFAFLHGNPWLCNCEILYFRRWLQDNAENVYVWKQKVDVKAMTSNVASVQCDNSDKFPVYKYPGKGCPTLGDEGDTDLYDYYPEEDTEGDKVRATRTVVKFPTKAHTTPWGLFYSWSTASLDSQMPSSLHPTQESTKEQTTFPPRWTPNFTLHMESITFSKTPKSTTEPTPSPTTSEPVPEPAPNMTTLEPTPSPTTPEPTSEPAPSPTTPEPTSEPAPSPTTPEPTSEPAPSPTTPEPTPIPTIATSPTILVSATSLITPKSTFLTTTKPVSLLESTKKTIPELDQPPKLRGVLQGHLESSRNDPFLHPDFTTTPAPRPPTPAPTIASQPLSLRPEACRPAAGGAVHTRGLDFACDIYIWAPLAGTCGVLLLSLVITLYCKRGRKKLLYIFKQPFMRPVQTTQEEDGCSCRFPEEEEGGCELRVKFSRSADAPAYQQGQNQLYNELNLGRREEYDVLDKRRGRDPEMGGKPRRKNPQEGLYNELQKDKMAEAYSEIGMKGERRRGKGHDGLYQGLSTATKDTYDALHMQALPPR

SEQ ID NO: 15 - protein, 637 aa, synthetic construct
HPICEVSKVASHLEVNCDKRNLTALPPDLPKDTTILHLSENLLYTFSLATLMPYTRLTQLNLDRCELTKLQVDGTLPVLGTLDLSHNQLQSLPLLGQTLPALTVLDVSFNRLTSLPLGALRGLGELQELYLKGNELKTLPPGLLTPTPKLEKLSLANNNLTELPAGLLNGLENLDTLLLQENSLYTIPKGFFGSHLLPFAFLHGNPWLCNCEILYFRRWLQDNAENVYVWKQKVDVKAMTSNVASVQCDNSDKFPVYKYPGKGCPTLGDEGDTDLYDYYPEEDTEGDKVRATRTVVKFPTKAHTTPWGLFYSWSTASLDSQMPSSLHPTQESTKEQTTFPPRWTPNFTLHMESITFSKTPKSTTEPTPSPTTSEPVPEPAPNMTTLEPTPSPTTPEPTSEPAPSPTTPEPTSEPTTTPAPRPPTPAPTIASQPLSLRPEACRPAAGGAVHTRGLDFACDIYIWAPLAGTCGVLLLSLVITLYCKRGRKKLLYIFKQPFMRPVQTTQEEDGCSCRFPEEEEGGCELRVKFSRSADAPAYQQGQNQLYNELNLGRREEYDVLDKRRGRDPEMGGKPRRKNPQEGLYNELQKDKMAEAYSEIGMKGERRRGKGHDGLYQGLSTATKDTYDALHMQALPPR

SEQ ID NO: 16 - DNA, 933 bp, synthetic construct
  source 1..933: mol_type = other DNA
atggccctgcccgtgaccgccctgctgctgcccctggccctgctgctgcacgccgcccgcccccaccccatctgtgaggtctccaaagtggccagccacctagaagtgaactgtgacaagaggaatctgacagcgctgcctccagacctgccgaaagacacaaccatcctccacctgagtgagaacctcctgtacaccttctccctggcaaccctgatgccttacactcgcctcactcagctgaacctagataggtgcgagctcaccaagctccaggtcgatgggacgctgccagtgctggggaccctggatctatcccacaatcagctgcaaagcctgcccttgctagggcagacactgcctgctctcaccgtcctggacgtctccttcaaccggctgacctcgctgcctcttggtgccctgcgtggtcttggcgaactccaagagctctacctgaaaggcaatgagctgaagaccctgcccccagggctcctgacgcccacacccaagctggagaagctcagtctggctaacaacaacttgactgagctccccgctgggctcctgaatgggctggagaatctcgacacccttctcctccaagagaactcgctgtatacaataccaaagggcttttttgggtcccacctcctgccttttgcttttctccacgggaacccctggttatgcaactgtgagatcctctattttcgtcgctggctgcaggacaatgctgaaaatgtctacgtatggaagcaaaaggtggacgtcaaggccatgacctctaacgtggccagtgtgcagtgtgacaattcagacaagtttcccgtctacaaatacccaggaaaggggtgccccacccttggtgatgaaggtgacacagacctatatgattactacccagaagaggacactgagggcgataaggtgcgt

SEQ ID NO: 17 - protein, 290 aa, synthetic construct
HPICEVSKVASHLEVNCDKRNLTALPPDLPKDTTILHLSENLLYTFSLATLMPYTRLTQLNLDRCELTKLQVDGTLPVLGTLDLSHNQLQSLPLLGQTLPALTVLDVSFNRLTSLPLGALRGLGELQELYLKGNELKTLPPGLLTPTPKLEKLSLANNNLTELPAGLLNGLENLDTLLLQENSLYTIPKGFFGSHLLPFAFLHGNPWLCNCEILYFRRWLQDNAENVYVWKQKVDVKAMTSNVASVQCDNSDKFPVYKYPGKGCPTLGDEGDTDLYDYYPEEDTEGDKVR

SEQ ID NO: 18 - DNA, 1590 bp, synthetic construct
  source 1..1590: mol_type = other DNA
atggccctgcccgtgaccgccctgctgctgcccctggccctgctgctgcacgccgcccgcccccaccccatctgtgaggtctccaaagtggccagccacctagaagtgaactgtgacaagaggaatctgacagcgctgcctccagacctgccgaaagacacaaccatcctccacctgagtgagaacctcctgtacaccttctccctggcaaccctgatgccttacactcgcctcactcagctgaacctagataggtgcgagctcaccaagctccaggtcgatgggacgctgccagtgctggggaccctggatctatcccacaatcagctgcaaagcctgcccttgctagggcagacactgcctgctctcaccgtcctggacgtctccttcaaccggctgacctcgctgcctcttggtgccctgcgtggtcttggcgaactccaagagctctacctgaaaggcaatgagctgaagaccctgcccccagggctcctgacgcccacacccaagctggagaagctcagtctggctaacaacaacttgactgagctccccgctgggctcctgaatgggctggagaatctcgacacccttctcctccaagagaactcgctgtatacaataccaaagggcttttttgggtcccacctcctgccttttgcttttctccacgggaacccctggttatgcaactgtgagatcctctattttcgtcgctggctgcaggacaatgctgaaaatgtctacgtatggaagcaaaaggtggacgtcaaggccatgacctctaacgtggccagtgtgcagtgtgacaattcagacaagtttcccgtctacaaatacccaggaaaggggtgccccacccttggtgatgaaggtgacacagacctatatgattactacccagaagaggacactgagggcgataaggtgcgtgccacaaggactgtggtcaagttccccaccaaagcccatacaaccccctggggtctattctactcatggtccactgcttctctagacagccaaatgccctcctccttgcatccaacacaagaatccactaaggagcagaccacattcccacctagatggaccccaaatttcacacttcacatggaatccatcacattctccaaaactccaaaatccactactgaaccaaccccaagcccgaccacctcagagcccgtcccggagcccgccccaaacatgaccaccctggagcccactccaagcccgaccaccccagagcccacctcagagcccgcccccagcccgaccaccccggagcccacctcagagcccgcccccagcccgaccaccccagagcccacctcagagcccgcccccagcccgaccaccccggagcccaccccaatcccgaccatcgccacaagcccgaccatcctggtgtctgccacaagcctgatcactccaaaaagcacatttttaactaccacaaaacccgtatcactcttagaatccaccaaaaaaaccatccctgaacttgatcagccaccaaagctccgtggggtgctccaagggcatttggagagctccagaaatgacccttttctccaccccgacttt

SEQ ID NO: 19 - protein, 509 aa, synthetic construct
HPICEVSKVASHLEVNCDKRNLTALPPDLPKDTTILHLSENLLYTFSLATLMPYTRLTQLNLDRCELTKLQVDGTLPVLGTLDLSHNQLQSLPLLGQTLPALTVLDVSFNRLTSLPLGALRGLGELQELYLKGNELKTLPPGLLTPTPKLEKLSLANNNLTELPAGLLNGLENLDTLLLQENSLYTIPKGFFGSHLLPFAFLHGNPWLCNCEILYFRRWLQDNAENVYVWKQKVDVKAMTSNVASVQCDNSDKFPVYKYPGKGCPTLGDEGDTDLYDYYPEEDTEGDKVRATRTVVKFPTKAHTTPWGLFYSWSTASLDSQMPSSLHPTQESTKEQTTFPPRWTPNFTLHMESITFSKTPKSTTEPTPSPTTSEPVPEPAPNMTTLEPTPSPTTPEPTSEPAPSPTTPEPTSEPAPSPTTPEPTSEPAPSPTTPEPTPIPTIATSPTILVSATSLITPKSTFLTTTKPVSLLESTKKTIPELDQPPKLRGVLQGHLESSRNDPFLHPDF

SEQ ID NO: 20 - DNA, 1305 bp, synthetic construct
  source 1..1305: mol_type = other DNA
atggccctgcccgtgaccgccctgctgctgcccctggccctgctgctgcacgccgcccgcccccaccccatctgtgaggtctccaaagtggccagccacctagaagtgaactgtgacaagaggaatctgacagcgctgcctccagacctgccgaaagacacaaccatcctccacctgagtgagaacctcctgtacaccttctccctggcaaccctgatgccttacactcgcctcactcagctgaacctagataggtgcgagctcaccaagctccaggtcgatgggacgctgccagtgctggggaccctggatctatcccacaatcagctgcaaagcctgcccttgctagggcagacactgcctgctctcaccgtcctggacgtctccttcaaccggctgacctcgctgcctcttggtgccctgcgtggtcttggcgaactccaagagctctacctgaaaggcaatgagctgaagaccctgcccccagggctcctgacgcccacacccaagctggagaagctcagtctggctaacaacaacttgactgagctccccgctgggctcctgaatgggctggagaatctcgacacccttctcctccaagagaactcgctgtatacaataccaaagggcttttttgggtcccacctcctgccttttgcttttctccacgggaacccctggttatgcaactgtgagatcctctattttcgtcgctggctgcaggacaatgctgaaaatgtctacgtatggaagcaaaaggtggacgtcaaggccatgacctctaacgtggccagtgtgcagtgtgacaattcagacaagtttcccgtctacaaatacccaggaaaggggtgccccacccttggtgatgaaggtgacacagacctatatgattactacccagaagaggacactgagggcgataaggtgcgtgccacaaggactgtggtcaagttccccaccaaagcccatacaaccccctggggtctattctactcatggtccactgcttctctagacagccaaatgccctcctccttgcatccaacacaagaatccactaaggagcagaccacattcccacctagatggaccccaaatttcacacttcacatggaatccatcacattctccaaaactccaaaatccactactgaaccaaccccaagcccgaccacctcagagcccgtcccggagcccgccccaaacatgaccaccctggagcccactccaagcccgaccaccccagagcccacctcagagcccgcccccagcccgaccaccccggagcccacctcagagccc

SEQ ID NO: 21 - protein, 414 aa, synthetic construct
HPICEVSKVASHLEVNCDKRNLTALPPDLPKDTTILHLSENLLYTFSLATLMPYTRLTQLNLDRCELTKLQVDGTLPVLGTLDLSHNQLQSLPLLGQTLPALTVLDVSFNRLTSLPLGALRGLGELQELYLKGNELKTLPPGLLTPTPKLEKLSLANNNLTELPAGLLNGLENLDTLLLQENSLYTIPKGFFGSHLLPFAFLHGNPWLCNCEILYFRRWLQDNAENVYVWKQKVDVKAMTSNVASVQCDNSDKFPVYKYPGKGCPTLGDEGDTDLYDYYPEEDTEGDKVRATRTVVKFPTKAHTTPWGLFYSWSTASLDSQMPSSLHPTQESTKEQTTFPPRWTPNFTLHMESITFSKTPKSTTEPTPSPTTSEPVPEPAPNMTTLEPTPSPTTPEPTSEPAPSPTTPEPTSEP